European Patent Application EP 4 803 620 A1, published September 9, 2026. Title: Novel small CRISPR-Cas12. Applicant: ISHINO, Yoshizumi. The sequence listing filed with the application follows.

SEQUENCE LISTING (8 sequences)

SEQ ID NO: 1 - DNA, 3751 bp, unidentified
  source 1..3751: mol_type = unassigned DNA
cttgctttccacatgtcaacgcatggtaagcagtttcctgtagcaggtctgatagcacgataagctggatgcacacggcaaccttttaccaacagttctagaagctctattttatgaagtaattttttcatgtttcagtctccttcatttttacttgggtaaaaacctaccacaaaatctattccaaacatcgtacttgcaccaatactcacaagtcgtgttttcaaccatgatttcctcaaagggtttaccttctatcgagcagtatccaacctttctgtcatatgtcgttttaccagtgagttcacaaatggcttgcttgcctttgaactgttttgcaaatcgtgtcgcagctttaccttcgcttgtactgttttcagggcaatccaaaacagcaatacgaataggaactccttttacctcaaacgtatcaccgtcacgaacatgagttatagtgcctcgtaaaactgatgccgctcttttatcaaaccctgtttctgggtctgtatatccgatgcctagttcatccatatagttcagaaacaaaaacgcagaggcaataagtattactacaataaggtttgatgaaggactgaagtagcgtcttctccttggtctagcgttggatacaacccttacgccagttcgctttttgaatgccgcagtcgtatctttctttttgcctgacttcctgacaggtcttctgttccaaggtgacggtgggggtttctttgtcatatacttaactagtctttattcttcatctctttcatagcttgatcaagagatgtaaactttaggttctcagaaccacactcgtcacatttatttgagagatccataccttctggcagtgccatccaactgttatgactcagtaactgcatcttgagtggcataacatgtccacagtccaaacaatcagcatgatatggtttaattacggtcatctaaaacaatacctaaaaccttgttacaagatgatacaaacaccatcagctattgttttggcaagtatcctacaccttgatccagttaaacttttaagtatcatcttggtatggcaactcgagtctacaaatatggtctgatacctattggctaccctccgcaggaagctattgatgaactgtttagggctaataaactgtggaacactcttgttgctttacacaaagagcatttcgagagatgggaagatgccagacgtacggcatctattgaatactcagaaaagttagatgaactagaggttaaacaacaacagataatggatgcatttgatgccttgcgacaagtacggatggaagaaggcactaaagacgagagcaatccaaggctaaagttgcaaagagatgttattaacaggctcagagatgaacagagtgttatatttacagagttaaagcctcttcgaaatgcagccaataaactgatagatacaaaagagataaatgacatatttcgaaccaaggtaaacgctgcagcttcaaccaaaactaatggtctctataatccaacggctgatgaagttgtgagaaactttaaagaagcaagacaacgtatctttgccaatcctaagtctcagctacgtttccatcgttttgatggcactggctactacaactttagatttagacgtaaaggtgaaaaacaggatggtgtttggttctcagagttatttgctggtaacgcaaaagaagacaaacggttctcagtaattggtagagacgatagccacaagaagacacgtctacgattaagagctacgatgactggtggggcaaccaaggctagtaaagtatatcaagagtttgattggatattacatagagatatctcagaaaatgctcagatccaaaacggtaagatcctaagaacacgctctggcgataagtttaaatatgatctcgttttaacattacgaatacctgatactgaaactcttccaccaaacagccttaaaggcactattggtatagatgttggatttaggaagtctggtgataccgtacttgttgccactgttctgtcagatgaagttggagccaaaccattggagatcaaagcaccttcaaagatggtatctgctctggaacacgtcatagatttacagggtgaactagacgatgctgctaacgacttaggtaaagctattacaccactaatgaagcagcaccgtttagaagaggatcaccaaaagtatcgcttttgtaagtcaattacagacagacctgccaatgtgaccctgtcctatgaaaaagcgtataagctagcgatatggctaaaccacgaacctgatgctctacctaaagagattacggctaaagtcttcacgtggtggcgcagctacagtcgcaaatatagagagatacataacagaagacgcaagcagcttacgcaccgcaagcacttctacagagaagctgccgccagtattgttgcccaacaaaagttaattgttttggagaagattaatctagcacgttttgctgagaccaaagacaaaaacactaagctcaccaataaagccagagcgcaacggttcttaggttcagtgtcagagttaagagatgcaataaagaatgcagcggatagagaaggtgttccttacatagaggtgaatcctgcgtacacgtctaaaacatgctctgagtgtggtgctttaaataaagagttaaaggctgagaaggagtggacttgtcagtcatgtggtgtcgtacatgacagagatactaatgctgcgaataacttacaaaacatgggtaagcagtacttagattatgtaaaaaacaaagatgatgcggtaatagagtaagcaacagatgcagtttttagctagtccaaatcgtctttttgctatagataacaaggaggtattaacctatcagattaaggcccttgtgtagtggggtgtaactacaacttataactaaaccgcacgttacaataccaggattaaggcccttgtgtagtggggtgtaactacaactacctgatagagtgtaagaggtataaagcagattaaggcccctgtgtagtggtgtgtaactacaacgaggaatgacttgaccttgcgagtcataagattaaggcccctgtgtagtggggtgtaactacaactattgctgtgcttccgtcataatctgttgtgattaaggcccctgtgtagtggggtgtaactacaacgaggttactgatctcgtcacgttctctatcgattaaggcccctgtgcgttggggtgtaaacgcaacccgtgggtgttaacagcgttaaaacctttgagttacggcccttgtgtagtggggtgtaaacaaataggtgcttagtcataaaggctaggcatcttttgtttaagctatccagttaaaaaaccacatctgtgtaaagtgatatataccactacggatgccatgccagtggccctccaacacacctctaaaactttttgatgttcaggttctagggcaatcagtatctacaaatagagagtaccaatagagcaaggtctaagaggactatactatatagtaccaatagggttgtgttttatatttttggtactatactcccacaatgtctaagacgttaaagggaatatagatatgttaataggtgtagctaggacatccaccatagaacaagttgcagggttggatgcacaagtacaacaattaaaagaatatggctgtgaaaagattttccaagagcaagtatcaagcgttggtgagcgtgaacaattaaacgtag

SEQ ID NO: 2 - DNA, 1758 bp, unidentified
  source 1..1758: mol_type = unassigned DNA
atggcaactcgagtctacaaatatggtctgatacctattggctaccctccgcaggaagctattgatgaactgtttagggctaataaactgtggaacactcttgttgctttacacaaagagcatttcgagagatgggaagatgccagacgtacggcatctattgaatactcagaaaagttagatgaactagaggttaaacaacaacagataatggatgcatttgatgccttgcgacaagtacggatggaagaaggcactaaagacgagagcaatccaaggctaaagttgcaaagagatgttattaacaggctcagagatgaacagagtgttatatttacagagttaaagcctcttcgaaatgcagccaataaactgatagatacaaaagagataaatgacatatttcgaaccaaggtaaacgctgcagcttcaaccaaaactaatggtctctataatccaacggctgatgaagttgtgagaaactttaaagaagcaagacaacgtatctttgccaatcctaagtctcagctacgtttccatcgttttgatggcactggctactacaactttagatttagacgtaaaggtgaaaaacaggatggtgtttggttctcagagttatttgctggtaacgcaaaagaagacaaacggttctcagtaattggtagagacgatagccacaagaagacacgtctacgattaagagctacgatgactggtggggcaaccaaggctagtaaagtatatcaagagtttgattggatattacatagagatatctcagaaaatgctcagatccaaaacggtaagatcctaagaacacgctctggcgataagtttaaatatgatctcgttttaacattacgaatacctgatactgaaactcttccaccaaacagccttaaaggcactattggtatagatgttggatttaggaagtctggtgataccgtacttgttgccactgttctgtcagatgaagttggagccaaaccattggagatcaaagcaccttcaaagatggtatctgctctggaacacgtcatagatttacagggtgaactagacgatgctgctaacgacttaggtaaagctattacaccactaatgaagcagcaccgtttagaagaggatcaccaaaagtatcgcttttgtaagtcaattacagacagacctgccaatgtgaccctgtcctatgaaaaagcgtataagctagcgatatggctaaaccacgaacctgatgctctacctaaagagattacggctaaagtcttcacgtggtggcgcagctacagtcgcaaatatagagagatacataacagaagacgcaagcagcttacgcaccgcaagcacttctacagagaagctgccgccagtattgttgcccaacaaaagttaattgttttggagaagattaatctagcacgttttgctgagaccaaagacaaaaacactaagctcaccaataaagccagagcgcaacggttcttaggttcagtgtcagagttaagagatgcaataaagaatgcagcggatagagaaggtgttccttacatagaggtgaatcctgcgtacacgtctaaaacatgctctgagtgtggtgctttaaataaagagttaaaggctgagaaggagtggacttgtcagtcatgtggtgtcgtacatgacagagatactaatgctgcgaataacttacaaaacatgggtaagcagtacttagattatgtaaaaaacaaagatgatgcggtaatagagtaa

SEQ ID NO: 3 - protein, 585 aa, unidentified
MATRVYKYGLIPIGYPPQEAIDELFRANKLWNTLVALHKEHFERWEDARRTASIEYSEKLDELEVKQQQIMDAFDALRQVRMEEGTKDESNPRLKLQRDVINRLRDEQSVIFTELKPLRNAANKLIDTKEINDIFRTKVNAAASTKTNGLYNPTADEVVRNFKEARQRIFANPKSQLRFHRFDGTGYYNFRFRRKGEKQDGVWFSELFAGNAKEDKRFSVIGRDDSHKKTRLRLRATMTGGATKASKVYQEFDWILHRDISENAQIQNGKILRTRSGDKFKYDLVLTLRIPDTETLPPNSLKGTIGIDVGFRKSGDTVLVATVLSDEVGAKPLEIKAPSKMVSALEHVIDLQGELDDAANDLGKAITPLMKQHRLEEDHQKYRFCKSITDRPANVTLSYEKAYKLAIWLNHEPDALPKEITAKVFTWWRSYSRKYREIHNRRRKQLTHRKHFYREAAASIVAQQKLIVLEKINLARFAETKDKNTKLTNKARAQRFLGSVSELRDAIKNAADREGVPYIEVNPAYTSKTCSECGALNKELKAEKEWTCQSCGVVHDRDTNAANNLQNMGKQYLDYVKNKDDAVIE

SEQ ID NO: 4 - DNA, 32 bp, unidentified
  source 1..32: mol_type = unassigned DNA
aaggcccttgtgtagtggggtgtaactacaac

SEQ ID NO: 5 - DNA, 32 bp, unidentified
  source 1..32: mol_type = unassigned DNA
aaggcccctgtgtagtggtgtgtaactacaac

SEQ ID NO: 6 - DNA, 32 bp, unidentified
  source 1..32: mol_type = unassigned DNA
aaggcccctgtgtagtggggtgtaactacaac

SEQ ID NO: 7 - DNA, 32 bp, unidentified
  source 1..32: mol_type = unassigned DNA
aaggcccctgtgcgttggggtgtaaacgcaac

SEQ ID NO: 8 - DNA, 32 bp, unidentified
  source 1..32: mol_type = unassigned DNA
acggcccttgtgtagtggggtgtaaacaaata